European Patent Application EP 4 186 526 A1, published May 31, 2023. Title: Agents improving anti-cance drug resistance. Applicant: Y's AC Co., Ltd. JUNTENDO EDUCATIONAL FOUNDATION. The sequence listing filed with the application follows.

SEQUENCE LISTING (53 sequences)

SEQ ID NO: 1 - DNA, 429 bp, Artificial Sequence
  antibody VH
  CDS (1)..(429)
  sig_peptide (1)..(57)
atggacaggcttacttcttcattcctgctgctgattgtccctgcatatgtcttgtcccaagttactctaaaagagtctggccctgggatattgaagccctcacagaccctcagtctgacttgttctttttctgggtttgcactgagcacttctggtatgggtgtaggctggattcgtcagccttcagggaagggtctggagtggctggcacacatttggtgggatgatgataagtactataacccatccctgaagagccagttcataatctccaaggattcctccagaaataaggtattcctcaagatcaccagtgtggacactgcagatactgccacttattactgtgctcgaagcccgccggagtatggtaactacggtctttcctttgactactggggccaaggcacctctctcttagtctcttca

SEQ ID NO: 2 - protein, 143 aa, Artificial Sequence
  Synthetic Construct
MDRLTSSFLLLIVPAYVLSQVTLKESGPGILKPSQTLSLTCSFSGFALSTSGMGVGWIRQPSGKGLEWLAHIWWDDDKYYNPSLKSQFIISKDSSRNKVFLKITSVDTADTATYYCARSPPEYGNYGLSFDYWGQGTSLLVSS

SEQ ID NO: 3 - DNA, 393 bp, Artificial Sequence
  antibody VL
  CDS (1)..(393)
  sig_peptide (1)..(57)
atgaagttgcctgttaggctgttggtgctgatgttctggattcctgcttccagcagtgatgttttgatgacccaaattccactctccctgcctgtcagtcttggagatcaagcctccatctcttgcagatctagtcagaacattgtatatagtaatggaaatacctatttagaatggtacctgcagaaaccaggccagtctccaaagctcctgatctacaaagtctccaaccgattttctggggtcccagacaggttcagtggcagtggatcagggacagatttcacactcaagattagtagagtggaggctgaggatctgggagtttattactgctttcaaggttcacatgttccgtggacgttcggtggaggcaccaagctggaaatcaaa

SEQ ID NO: 4 - protein, 131 aa, Artificial Sequence
  Synthetic Construct
MKLPVRLLVLMFWIPASSSDVLMTQIPLSLPVSLGDQASISCRSSQNIVYSNGNTYLEWYLQKPGQSPKLLIYKVSNRFSGVPDRFSGSGSGTDFTLKISRVEAEDLGVYYCFQGSHVPWTFGGGTKLEIK

SEQ ID NO: 5 - protein, 7 aa, Artificial Sequence
  CDRH
TSGMGVG

SEQ ID NO: 6 - protein, 16 aa, Artificial Sequence
  CDRH
HIWWDDDKYYNPSLKS

SEQ ID NO: 7 - protein, 14 aa, Artificial Sequence
  CDRH
SPPEYGNYGLSFDY

SEQ ID NO: 8 - protein, 16 aa, Artificial Sequence
  CDRL
RSSQNIVYSNGNTYLE

SEQ ID NO: 9 - protein, 7 aa, Artificial Sequence
  CDRL
KVSNRFS

SEQ ID NO: 10 - protein, 9 aa, Artificial Sequence
  CDRL
FQGSHVPWT

SEQ ID NO: 11 - DNA, 426 bp, Artificial Sequence
  antibody VH
  sig_peptide (1)..(57)
  CDS (1)..(426)
atggacaggcttacttcttcattcctgctgctgattgtccctgcatatgtcttgtcccaagttactctaaaagagtctggccctggaatattgaagccctcacagaccctcagtctgacttgttctttctctgggttttcactgagcacttctggtatgggtgtaggctggattcgtcagccttcagggaagggtctggagtggctggcacacatttggtgggatgatgataagtactataacccatccctgaagagccaactcacaatctccaaggatacctccagaaaccaggtattcctcaagatcaccagtgtggacactgcagatactgccacttactactgtgttcgtggtggcattactgcgactcattactatgctatggactactggggtcaaggaacctcagtcaccgtctcctca

SEQ ID NO: 12 - protein, 142 aa, Artificial Sequence
  Synthetic Construct
MDRLTSSFLLLIVPAYVLSQVTLKESGPGILKPSQTLSLTCSFSGFSLSTSGMGVGWIRQPSGKGLEWLAHIWWDDDKYYNPSLKSQLTISKDTSRNQVFLKITSVDTADTATYYCVRGGITATHYYAMDYWGQGTSVTVSS

SEQ ID NO: 13 - DNA, 381 bp, Artificial Sequence
  antibody VL
  CDS (1)..(381)
  sig_peptide (1)..(60)
atgaacatgctcactcagctcctgggattactgctgctctggtttgcaggtggtaaatgtgacattcagatgacccagtctcctgcctcccagtctgcatctctgggagaaagtgtcaccatctcatgcctggcaagtcagaccattggtacatggttatcatggtatcagcagaaaccagggaaatctcctcagctcctgatttatgctgcaaccagcttggcagatggggtcccatcaaggttcagtggtagtggatctggcacaaaattttctttcaagatcagcagcctacaggctgaagattttgtaagttattactgtcaacaactttacagtagtccgtggacgttcggtggaggcaccaagctggaaatcaaa

SEQ ID NO: 14 - protein, 127 aa, Artificial Sequence
  Synthetic Construct
MNMLTQLLGLLLLWFAGGKCDIQMTQSPASQSASLGESVTISCLASQTIGTWLSWYQQKPGKSPQLLIYAATSLADGVPSRFSGSGSGTKFSFKISSLQAEDFVSYYCQQLYSSPWTFGGGTKLEIK

SEQ ID NO: 15 - protein, 7 aa, Artificial Sequence
  CDRH
TSGMGVG

SEQ ID NO: 16 - protein, 16 aa, Artificial Sequence
  CDRH
HIWWDDDKYYNPSLKS

SEQ ID NO: 17 - protein, 13 aa, Artificial Sequence
  CDRH
GGITATHYYAMDY

SEQ ID NO: 18 - protein, 11 aa, Artificial Sequence
  CDRL
LASQTIGTWLS

SEQ ID NO: 19 - protein, 7 aa, Artificial Sequence
  CDRL
AATSLAD

SEQ ID NO: 20 - protein, 9 aa, Artificial Sequence
  CDRL
QQLYSSPWT

SEQ ID NO: 21 - DNA, 463 bp, Artificial Sequence
  heavy chain variable region
actagtgccaccatggacaggcttacttcttcattcctgctgctgattgtccctgcatatgtcttgtcccaagttactctgaaagagtctggccctgcactcgtgaagcccacacagaccctcactctgacttgtactttctctgggttttcactgagcacttctggcatgggcgtcggctggattcgtcagcctccagggaaggcactggagtggctggcacacatttggtgggatgatgataagtactataacccatccctgaagagccaactcacaatctccaaggatacctccaaaaaccaagtggtcctcaccatgaccaatatggaccctgttgatactgccacttactactgtgttcgtggaggcattactgccactcattactatgctatggactactggggtcaaggaaccacagtcaccgtctcctcaggtaagtatggcctctccaaagctt

SEQ ID NO: 22 - DNA, 426 bp, Artificial Sequence
  heavy chain variable region
  CDS (1)..(426)
  sig_peptide (1)..(426)
atggacaggcttacttcttcattcctgctgctgattgtccctgcatatgtcttgtcccaagttactctgaaagagtctggccctgcactcgtgaagcccacacagaccctcactctgacttgtactttctctgggttttcactgagcacttctggcatgggcgtcggctggattcgtcagcctccagggaaggcactggagtggctggcacacatttggtgggatgatgataagtactataacccatccctgaagagccaactcacaatctccaaggatacctccaaaaaccaagtggtcctcaccatgaccaatatggaccctgttgatactgccacttactactgtgttcgtggaggcattactgccactcattactatgctatggactactggggtcaaggaaccacagtcaccgtctcctca

SEQ ID NO: 23 - protein, 142 aa, Artificial Sequence
  Synthetic Construct
MDRLTSSFLLLIVPAYVLSQVTLKESGPALVKPTQTLTLTCTFSGFSLSTSGMGVGWIRQPPGKALEWLAHIWWDDDKYYNPSLKSQLTISKDTSKNQVVLTMTNMDPVDTATYYCVRGGITATHYYAMDYWGQGTTVTVSS

SEQ ID NO: 24 - DNA, 369 bp, Artificial Sequence
  heavy chain variable region
  CDS (1)..(369)
caagttactctgaaagagtctggccctgcactcgtgaagcccacacagaccctcactctgacttgtactttctctgggttttcactgagcacttctggcatgggcgtcggctggattcgtcagcctccagggaaggcactggagtggctggcacacatttggtgggatgatgataagtactataacccatccctgaagagccaactcacaatctccaaggatacctccaaaaaccaagtggtcctcaccatgaccaatatggaccctgttgatactgccacttactactgtgttcgtggaggcattactgccactcattactatgctatggactactggggtcaaggaaccacagtcaccgtctcctca

SEQ ID NO: 25 - protein, 123 aa, Artificial Sequence
  Synthetic Construct
QVTLKESGPALVKPTQTLTLTCTFSGFSLSTSGMGVGWIRQPPGKALEWLAHIWWDDDKYYNPSLKSQLTISKDTSKNQVVLTMTNMDPVDTATYYCVRGGITATHYYAMDYWGQGTTVTVSS

SEQ ID NO: 26 - DNA, 418 bp, Artificial Sequence
  light chain variable region
gctagcgccaccatgaacatgctcactcagctcctgggacttctgctgctctggtttgcaggcggaaaatgtgacattcagatgacccagtctccttcctccctgtctgcatctgtgggagacagagtcaccatcacatgcctggcaagtcagaccattggcacatggctgtcatggtatcagcagaaaccagggaaagctcctaagctcctgatttatgctgcaaccagcttggcagatggggtcccatcaagattcagtggaagtggatctggcacaaagtttaccttcaccatcagcagcctgcagcctgaagatattgccacttattactgtcaacagctttacagtagtccctggactttcggaggaggcaccaaagtcgaaatcaaacgtaagtagaatccaaagtgaattc

SEQ ID NO: 27 - DNA, 381 bp, Artificial Sequence
  light chain variable region
  CDS (1)..(381)
  sig_peptide (1)..(381)
atgaacatgctcactcagctcctgggacttctgctgctctggtttgcaggcggaaaatgtgacattcagatgacccagtctccttcctccctgtctgcatctgtgggagacagagtcaccatcacatgcctggcaagtcagaccattggcacatggctgtcatggtatcagcagaaaccagggaaagctcctaagctcctgatttatgctgcaaccagcttggcagatggggtcccatcaagattcagtggaagtggatctggcacaaagtttaccttcaccatcagcagcctgcagcctgaagatattgccacttattactgtcaacagctttacagtagtccctggactttcggaggaggcaccaaagtcgaaatcaaa

SEQ ID NO: 28 - protein, 127 aa, Artificial Sequence
  Synthetic Construct
MNMLTQLLGLLLLWFAGGKCDIQMTQSPSSLSASVGDRVTITCLASQTIGTWLSWYQQKPGKAPKLLIYAATSLADGVPSRFSGSGSGTKFTFTISSLQPEDIATYYCQQLYSSPWTFGGGTKVEIK

SEQ ID NO: 29 - DNA, 321 bp, Artificial Sequence
  light chain variable region
  CDS (1)..(321)
gacattcagatgacccagtctccttcctccctgtctgcatctgtgggagacagagtcaccatcacatgcctggcaagtcagaccattggcacatggctgtcatggtatcagcagaaaccagggaaagctcctaagctcctgatttatgctgcaaccagcttggcagatggggtcccatcaagattcagtggaagtggatctggcacaaagtttaccttcaccatcagcagcctgcagcctgaagatattgccacttattactgtcaacagctttacagtagtccctggactttcggaggaggcaccaaagtcgaaatcaaa

SEQ ID NO: 30 - protein, 107 aa, Artificial Sequence
  Synthetic Construct
DIQMTQSPSSLSASVGDRVTITCLASQTIGTWLSWYQQKPGKAPKLLIYAATSLADGVPSRFSGSGSGTKFTFTISSLQPEDIATYYCQQLYSSPWTFGGGTKVEIK

SEQ ID NO: 31 - DNA, 418 bp, Artificial Sequence
  light chain variable region
gctagcgccaccatgaacatgctcactcagctcctgggacttctgctgctctggtttgcaggcggaaaatgtgacattcagatgacccagtctccttcctccctgtctgcatctgtgggagacagagtcaccatcacatgcctggcaagtcagaccattggcacatggctgtcatggtatcagcagaaaccagggaaagctcctaagctcctgatttatgctgcaaccagcttggcagatggggtcccatcaagattcagtggaagtggatctggcacagactttaccttcaccatcagcagcctgcagcctgaagatattgccacttattactgtcaacagctttacagtagtccctggactttcggaggaggcaccaaagtcgaaatcaaacgtaagtagaatccaaagtgaattc

SEQ ID NO: 32 - DNA, 381 bp, Artificial Sequence
  light chain variable region
  CDS (1)..(381)
  sig_peptide (1)..(381)
atgaacatgctcactcagctcctgggacttctgctgctctggtttgcaggcggaaaatgtgacattcagatgacccagtctccttcctccctgtctgcatctgtgggagacagagtcaccatcacatgcctggcaagtcagaccattggcacatggctgtcatggtatcagcagaaaccagggaaagctcctaagctcctgatttatgctgcaaccagcttggcagatggggtcccatcaagattcagtggaagtggatctggcacagactttaccttcaccatcagcagcctgcagcctgaagatattgccacttattactgtcaacagctttacagtagtccctggactttcggaggaggcaccaaagtcgaaatcaaa

SEQ ID NO: 33 - protein, 127 aa, Artificial Sequence
  Synthetic Construct
MNMLTQLLGLLLLWFAGGKCDIQMTQSPSSLSASVGDRVTITCLASQTIGTWLSWYQQKPGKAPKLLIYAATSLADGVPSRFSGSGSGTDFTFTISSLQPEDIATYYCQQLYSSPWTFGGGTKVEIK

SEQ ID NO: 34 - DNA, 321 bp, Artificial Sequence
  light chain variable region
  CDS (1)..(321)
gacattcagatgacccagtctccttcctccctgtctgcatctgtgggagacagagtcaccatcacatgcctggcaagtcagaccattggcacatggctgtcatggtatcagcagaaaccagggaaagctcctaagctcctgatttatgctgcaaccagcttggcagatggggtcccatcaagattcagtggaagtggatctggcacagactttaccttcaccatcagcagcctgcagcctgaagatattgccacttattactgtcaacagctttacagtagtccctggactttcggaggaggcaccaaagtcgaaatcaaa

SEQ ID NO: 35 - protein, 107 aa, Artificial Sequence
  Synthetic Construct
DIQMTQSPSSLSASVGDRVTITCLASQTIGTWLSWYQQKPGKAPKLLIYAATSLADGVPSRFSGSGSGTDFTFTISSLQPEDIATYYCQQLYSSPWTFGGGTKVEIK

SEQ ID NO: 36 - DNA, 1419 bp, Artificial Sequence
  heavy chain
  CDS (1)..(1416)
  sig_peptide (1)..(57)
atggacaggcttacttcttcattcctgctgctgattgtccctgcatatgtcttgtcccaagttactctgaaagagtctggccctgcactcgtgaagcccacacagaccctcactctgacttgtactttctctgggttttcactgagcacttctggcatgggcgtcggctggattcgtcagcctccagggaaggcactggagtggctggcacacatttggtgggatgatgataagtactataacccatccctgaagagccaactcacaatctccaaggatacctccaaaaaccaagtggtcctcaccatgaccaatatggaccctgttgatactgccacttactactgtgttcgtggaggcattactgccactcattactatgctatggactactggggtcaaggaaccacagtcaccgtctcctcagcctccaccaagggcccatcggtcttccccctggcaccctcctccaagagcacctctgggggcacagcggccctgggctgcctggtcaaggactacttccccgaaccggtgacggtgtcgtggaactcaggcgccctgaccagcggcgtgcacaccttcccggctgtcctacagtcctcaggactctactccctcagcagcgtggtgaccgtgccctccagcagcttgggcacccagacctacatctgcaacgtgaatcacaagcccagcaacaccaaggtggacaagaaagttgagcccaaatcttgtgacaaaactcacacatgcccaccgtgcccagcacctgaactcctggggggaccgtcagtcttcctcttccccccaaaacccaaggacaccctcatgatctcccggacccctgaggtcacatgcgtggtggtggacgtgagccacgaagaccctgaggtcaagttcaactggtacgtggacggcgtggaggtgcataatgccaagacaaagccgcgggaggagcagtacaacagcacgtaccgtgtggtcagcgtcctcaccgtcctgcaccaggactggctgaatggcaaggagtacaagtgcaaggtctccaacaaagccctcccagcccccatcgagaaaaccatctccaaagccaaagggcagccccgagaaccacaggtgtacaccctgcccccatcccgggatgagctgaccaagaaccaggtcagcctgacctgcctggtcaaaggcttctatcccagcgacatcgccgtggagtgggagagcaatgggcagccggagaacaactacaagaccacgcctcccgtgctggactccgacggctccttcttcctctacagcaagctcaccgtggacaagagcaggtggcagcaggggaacgtcttctcatgctccgtgatgcatgaggctctgcacaaccactacacgcagaagagcctctccctgtctccgggtaaatga

SEQ ID NO: 37 - protein, 472 aa, Artificial Sequence
  Synthetic Construct
MDRLTSSFLLLIVPAYVLSQVTLKESGPALVKPTQTLTLTCTFSGFSLSTSGMGVGWIRQPPGKALEWLAHIWWDDDKYYNPSLKSQLTISKDTSKNQVVLTMTNMDPVDTATYYCVRGGITATHYYAMDYWGQGTTVTVSSASTKGPSVFPLAPSSKSTSGGTAALGCLVKDYFPEPVTVSWNSGALTSGVHTFPAVLQSSGLYSLSSVVTVPSSSLGTQTYICNVNHKPSNTKVDKKVEPKSCDKTHTCPPCPAPELLGGPSVFLFPPKPKDTLMISRTPEVTCVVVDVSHEDPEVKFNWYVDGVEVHNAKTKPREEQYNSTYRVVSVLTVLHQDWLNGKEYKCKVSNKALPAPIEKTISKAKGQPREPQVYTLPPSRDELTKNQVSLTCLVKGFYPSDIAVEWESNGQPENNYKTTPPVLDSDGSFFLYSKLTVDKSRWQQGNVFSCSVMHEALHNHYTQKSLSLSPGK

SEQ ID NO: 38 - DNA, 705 bp, Artificial Sequence
  light chain
  CDS (1)..(702)
  sig_peptide (1)..(60)
atgaacatgctcactcagctcctgggacttctgctgctctggtttgcaggcggaaaatgtgacattcagatgacccagtctccttcctccctgtctgcatctgtgggagacagagtcaccatcacatgcctggcaagtcagaccattggcacatggctgtcatggtatcagcagaaaccagggaaagctcctaagctcctgatttatgctgcaaccagcttggcagatggggtcccatcaagattcagtggaagtggatctggcacaaagtttaccttcaccatcagcagcctgcagcctgaagatattgccacttattactgtcaacagctttacagtagtccctggactttcggaggaggcaccaaagtcgaaatcaaacgaactgtggctgcaccatctgtcttcatcttcccgccatctgatgagcagttgaaatctggaactgcctctgttgtgtgcctgctgaataacttctatcccagagaggccaaagtacagtggaaggtggataacgccctccaatcgggtaactcccaggagagtgtcacagagcaggacagcaaggacagcacctacagcctcagcagcaccctgacgctgagcaaagcagactacgagaaacacaaagtctacgcctgcgaagtcacccatcagggcctgagctcgcccgtcacaaagagcttcaacaggggagagtgttag

SEQ ID NO: 39 - protein, 234 aa, Artificial Sequence
  Synthetic Construct
MNMLTQLLGLLLLWFAGGKCDIQMTQSPSSLSASVGDRVTITCLASQTIGTWLSWYQQKPGKAPKLLIYAATSLADGVPSRFSGSGSGTKFTFTISSLQPEDIATYYCQQLYSSPWTFGGGTKVEIKRTVAAPSVFIFPPSDEQLKSGTASVVCLLNNFYPREAKVQWKVDNALQSGNSQESVTEQDSKDSTYSLSSTLTLSKADYEKHKVYACEVTHQGLSSPVTKSFNRGEC

SEQ ID NO: 40 - DNA, 705 bp, Artificial Sequence
  light chain
  CDS (1)..(702)
  sig_peptide (1)..(60)
atgaacatgctcactcagctcctgggacttctgctgctctggtttgcaggcggaaaatgtgacattcagatgacccagtctccttcctccctgtctgcatctgtgggagacagagtcaccatcacatgcctggcaagtcagaccattggcacatggctgtcatggtatcagcagaaaccagggaaagctcctaagctcctgatttatgctgcaaccagcttggcagatggggtcccatcaagattcagtggaagtggatctggcacagactttaccttcaccatcagcagcctgcagcctgaagatattgccacttattactgtcaacagctttacagtagtccctggactttcggaggaggcaccaaagtcgaaatcaaacgaactgtggctgcaccatctgtcttcatcttcccgccatctgatgagcagttgaaatctggaactgcctctgttgtgtgcctgctgaataacttctatcccagagaggccaaagtacagtggaaggtggataacgccctccaatcgggtaactcccaggagagtgtcacagagcaggacagcaaggacagcacctacagcctcagcagcaccctgacgctgagcaaagcagactacgagaaacacaaagtctacgcctgcgaagtcacccatcagggcctgagctcgcccgtcacaaagagcttcaacaggggagagtgttag

SEQ ID NO: 41 - protein, 234 aa, Artificial Sequence
  Synthetic Construct
MNMLTQLLGLLLLWFAGGKCDIQMTQSPSSLSASVGDRVTITCLASQTIGTWLSWYQQKPGKAPKLLIYAATSLADGVPSRFSGSGSGTDFTFTISSLQPEDIATYYCQQLYSSPWTFGGGTKVEIKRTVAAPSVFIFPPSDEQLKSGTASVVCLLNNFYPREAKVQWKVDNALQSGNSQESVTEQDSKDSTYSLSSTLTLSKADYEKHKVYACEVTHQGLSSPVTKSFNRGEC

SEQ ID NO: 42 - protein, 87 aa, Homo sapiens
QVTLKESGPALVKPTQTLTLTCTFSGFSLSWIRQPPGKALEWLARLTISKDTSKNQVVLTMTNMDPVDTATYYCARWGQGTTVTVSS

SEQ ID NO: 43 - protein, 80 aa, Homo sapiens
DIQMTQSPSSLSASVGDRVTITCWYQQKPGKAPKLLIYGVPSRFSGSGSGTDFTFTISSLQPEDIATYYCFGGGTKVEIK

SEQ ID NO: 44 - protein, 123 aa, Mus musculus
QVTLKESGPGILKPSQTLSLTCSFSGFSLSTSGMGVGWIRQPSGKGLEWLAHIWWDDDKYYNPSLKSQLTISKDTSRNQVFLKITSVDTADTATYYCVRGGITATHYYAMDYWGQGTSVTVSS

SEQ ID NO: 45 - protein, 107 aa, Mus musculus
DIQMTQSPASQSASLGESVTISCLASQTIGTWLSWYQQKPGKSPQLLIYAATSLADGVPSRFSGSGSGTKFSFKISSLQAEDFVSYYCQQLYSSPWTFGGGTKLEIK

SEQ ID NO: 46 - DNA, 20 bp, Artificial Sequence
  primer
gccagtggatagacagatgg

SEQ ID NO: 47 - DNA, 21 bp, Artificial Sequence
  primer
gatggatacagttggtgcagc

SEQ ID NO: 48 - DNA, 24 bp, Artificial Sequence
  primer
gaaccgtcagatcgcctggagacg

SEQ ID NO: 49 - DNA, 20 bp, Artificial Sequence
  primer
tgaaagatgagctggaggac

SEQ ID NO: 50 - DNA, 20 bp, Artificial Sequence
  primer
ctttcttgtccaccttggtg

SEQ ID NO: 51 - DNA, 19 bp, Artificial Sequence
  primer
gctgtcctacagtcctcag

SEQ ID NO: 52 - DNA, 18 bp, Artificial Sequence
  primer
acgtgccaagcatcctcg

SEQ ID NO: 53 - DNA, 18 bp, Artificial Sequence
  primer
ctgaggtcacatgcgtgg